European Patent Application EP 4 772 528 A1, published July 8, 2026. Title: Peptide Having Activity of Skin Whitening and Uses Thereof. Applicant: CAREGEN CO., LTD. The sequence listing filed with the application follows.

SEQUENCE LISTING (7 sequences)

SEQ ID NO: 1 - protein, 5 aa, synthetic construct
HSDAV

SEQ ID NO: 2 - DNA, 20 bp, synthetic construct
  source 1..20: mol_type = other DNA
tgctagcagcctctctctcc

SEQ ID NO: 3 - DNA, 20 bp, synthetic construct
  source 1..20: mol_type = other DNA
cttcaaggggaaccagatga

SEQ ID NO: 4 - DNA, 20 bp, synthetic construct
  source 1..20: mol_type = other DNA
tgaccaaacgtatccccctg

SEQ ID NO: 5 - DNA, 20 bp, synthetic construct
  source 1..20: mol_type = other DNA
ggtgtctgccgttgaagaga

SEQ ID NO: 6 - DNA, 20 bp, synthetic construct
  source 1..20: mol_type = other DNA
ggagccaaaagggtcatcat

SEQ ID NO: 7 - DNA, 20 bp, synthetic construct
  source 1..20: mol_type = other DNA
gtgatggcatggactgtggt